European Patent Specification EP 4 258 865 B1, published September 3, 2025. Title: HEAVY CHAIN-ONLY ANTIBODIES. Applicant: Trianni, Inc. The sequence listing filed with the application follows.

SEQUENCE LISTING (18 sequences)

SEQ ID NO: 1 - DNA, 2182 bp, Artificial Sequence
  polynucleotide
agtcagcttctgatggaattagaacttggcaaaacaatactgagaatgaagtgtatgtggaacagaggctgctgatctcgttcttcaggctatgaaactgacacatttggaaaccacagtacttagaaccacaaagtgggaatcaagagaaaaacaatgatcccacgagagatctatagatctatagatcatgagtgggaggaatgagctggcccttaatttggttttgcttgtttaaattatgatatccaactatgaaacattatcataaagcaatagtaaagagccttcagtaaagagcaggcatttatctaatcccaccccacccccacccccgtagctccaatccttccattcaaaatgtaggtactctgttctcacccttcttaacaaagtatgacaggaaaaacttccattttagtggacatctttattgtttaatagatcatcaatttctgcagacttacaggacggatcgatcccctcagttagcctcccccatctcccgggcaaacgtgcgcgccaggtcgcatatcgtcggtatggagccgggggtggtgacgtgggtctggaccatcccggaggtaagttgcagcagggcgtcccggcagccggcgggcgattggtcgtaatccaggataaagacgtgcatggaacggaggcgtttggccaagacgtccaaggcccaggcaaacacgttatacaggtcgccgttgggggccagcaactcgggggcccgaaacagggtaaataacgtgtccccgatatggggtcgtgggcccgcgttgctctggggctcggcaccctggggcggcacggccgtccccgaaagctgtccccagtcctcccgccacgacccgccgcactgcagataccgcaccgtattggcaagtagcccgtaaacgcggcgaatcgcagccagcatagccaggtccagccgctcgccggggcgctggcgtttggccaggcggtcgatgtgtctgtcctccggaagggccccaagcacgatgttggtgccgggcaaggtcggcgggatgagggccacgaacgccagcacggcctggggggtcatgctgcccataaggtaccgcgcggccgggtagcacaggagggcggcgatgggatggcggtcgaagatgagggtgagggccgggggcggggcatgtgagctcccagcctcccccccgatatgaggagccagaacggcgtcggtcacggcataaggcatgcccattgttatctgggcgcttgtcattaccaccgccgcgtccccggccgatatctcaccctggtcgaggcggtgttgtgtggtgtagatgttcgcgattgtctcggaagcccccagcacccgccagtaagtcatcggctcgggtacgtagacgatatcgtcgcgcgaacccagggccaccagcagttgcgtggtggtggttttccccatcccgtggggaccgtctatataaacccgcagtagcgtgggcattttctgctccgggcggacttccgtggcttcttgctgccggcgagggcgcaacgccgtacgtcggttgctatggccgcgagaacgcgcagcctggtcgaacgcagacgcgtgttgatggccggggtacgaggccatgatggcaaggacggtgcattggctgcaggtcgaaaggcccggagatgaggaagaggagaacagcgcggcagacgtgcgcttttgaagcgtgcagaatgccgggcctccggaggaccttcgggcgcccgccccgcccctgagcccgcccctgagcccgcccccggacccaccccttcccagcctctgagcccagaaagcgaaggagcaaagctgctattggccgctgccccaaaggcctacccgcttccattgctcagcggtgctgtccatctgcacgagactagtgagacgtgctacttccatttgtcacgtcctgcacgacgcgagctgcggggcgggggggaacttcctgactaggggaggagtagaaggtggcgcgaaggggccaccaaagaacggagccggttggcgcctaccggtggatgtggaatgtgtgcgaggccagaggccacttgtgtagcgccaagtgcccagcggggctgctaaagcgcatgctccagactgccttgggaaaagcgcctcccctacccggtagaattgacctgccggggccctcgaatcctgcag

SEQ ID NO: 2 - DNA, 2369 bp, Artificial Sequence
  polynucleotide
aggtgctcagcaaaggaggtcggcaggagggcggagggtgtgtttttgtatgggagaagcaggagggcagaggctgtgggtttttgttataggaacagaggcagaacagacactgtgctactggtacttcgatctctggggccgtggcaccctggtcactgtctcctcaggtaagctggcttttttctttctgcacattccattctgaaacgggaaaagatattctcagatctccccatgtcaggccatctgccacactgtgagtcctgcatctggggactgtggggttcaggtggcctaaggcaggatgtggagaggtttttgttcggggaacagaggggtatccaacactgtgtgatgcttttgatatctggggccaagggacaatggtcaccgtctcttcaggtaagatggctttccttctgcctcctttctctgggcccagcgtcctctgtcctggagctgggagataatgtccgggggctccttggtctgcgctgggccatgtggggccctccggggctccttctccggctgtctgcatgctgcagaagcttttctgtaaggatagggtcttcactcccaggaaaagaggcagtcagaggctagctgcctgtggaacagtgacaatcatggaaaataggcatttacattgttaggctacatgggtagatgggtttttgtacacccactaaaggggtctatgacactgtgactactttgactactggggccagggaaccctggtcaccgtctcctcaggtgagtccttacaacctctctcttctattcagcttaaatagattttactgcatttgttgggggggaaatgtgtgtatctgaatttcaggtcatgaaggactagggacaccttgggagtcagaaagggtcattgggagccctggctgacgcagacagacatcctcagctcccatacttcatggccagagatttatagggatcctggccagcattgccgctaggtccctctcttctatgctttctttgtccctcactggcctccatctgagatcatcctggagccctagccaaggatcggtttttgtcaggggtctaatcattgttgtcacactgtgacaactggttcgacccctggggccagggaaccctggtcaccgtctcctcaggtgagtcctaacttctcccattctaaatgcatgttggggggattctgggccttcaggaccaagattctctgcaaacgggaatcaagattcaacccctttgtcccaaagttgagacatgggtctgggtcagggactctctgcctgctggtctgtggtgacattagaactgaagtatgatgaaggatctgccagaactgaagcttgaagtctgaggcagaatcttgtccagggtctatcggactcttgtgagaattaggggctgacagttgatggtgacaatttcagggtcagtgactgtctggtttctctgaggtgaggctggaatataggtcaccttgaagactaaagaggggtccaggggcttctgcacaggcagggaacagaatgtggaacaatgacttgaatggttgattcttgtgtgacaccaggaattggcataatgtctgagttgcccaggggtgattctagtcagactctgggtttttgttcgggtatagaggaaaaatccaccactgtgattactactactactactacatggacgtctggggcaaagggaccacggtcaccgtctcctcaggtaagaatggcctctccaggtctttatttttaacctttgttatggagttttctgagcattgcagactaatcttggatatttgtccctgagggagccggctgagagaagttgggaaataaactgtctagggatctcagagcctttaggacaaacggtggctgccgtcctgacaggggcttagggaggctccaggacctcagtgccttgaagctggtttccaagagaaaaggattgtttatcttaggaggcatgcttactgttaaaagacaggatatgtttgaagtggcttctgagaaaaatggttaagaaaattatgacttaaaaatgtgagagattttcaagtatattaatttttttaactgtccaagtatttgaaattcttatcatttgattaacacccatgagtgatatgtgtctggaattgaggccaaagcaagctcagctaagaaatactagcacagtgctgtcggccccgatgcgggactgcgttttgaccatcataaatcaagtttatttttttaattaattgagcgaagctggaagcagatgatgaattagagtcaagatggctgcatgggggtctccggcacccacagcaggtggcaggaagcaggtcaccgcgagagtctattttaggaagc

SEQ ID NO: 3 - DNA, 19 bp, Artificial Sequence
  polynucleotide
cctttagtgagggttaatt

SEQ ID NO: 4 - DNA, 48 bp, Artificial Sequence
  polynucleotide
gaagttcctattccgaagttcctattcttcaaaaggtataggaacttc

SEQ ID NO: 5 - DNA, 2711 bp, Artificial Sequence
  polynucleotide
tcattctggcctccccctcccccaaggtcattctggcctccccctcccccaaggtcattctggcctccccctcccccttggccgcgcctcattctggcctccccctcccccaaggcacacaaaaaaccaacacacagatctattgaaaataatgatcttttattgatccgcgcctggatctcgaaccggttcaggcaccgggcttgcgggtcatgcaccaggtgcgcggtccttcgggcacctcgacgtcggcggtgacggtgaagccgagccgctcgtagaaggggaggttgcggggcgcggaggtctccaggaaggcgggcaccccggcgcgctcggccgcctccactccggggagcacgacggcgctgcccagacccttgccctggtggtcgggcgagacgccgacggtggccaggaaccacgcgggctccttgggccggtgcggcgccaggaggccttccatctgttgctgcgcggccagccgggaaccgctcaactcggccatgcgcgggccgatctcggcgaacaccgcccccgcttcgacgctctccggcgtggtccagaccgccaccgcggcgccgtcgtccgcgacccacaccttgccgatgtcgagcccgacgcgcgtgaggaagagttcttgcagctcggtgacccgctcgatgtggcggtccgggtcgacggtgtggcgcgtggcggggtagtcggcgaacgcggcggcgagggtgcgtacggcccgggggacgtcgtcgcgggtggcgaggcgcaccgtgggcttgtactcggtcatggaaggctaggcggatcggcgatcgctccggaggccgccctgggagtggacacctgtggagagaaaggcaaagtggatgtcaatgtcactcaagtgtatggccagatctcaagcctgccacacctcaagcttgacaacaaaaagattgtcttttctgaccagatggacgcggccaccctcaaaggcatcaccgcgggccaggtgaatatcaaatcctcctcgtttttggaaactgacaatcttagcgcagaagtcatgcccgcttttgagagggagtactcaccccaacgcttctagagccgccggtcacacgccagaagccgaaccccgccctgccccgtcccccccgaaggcagccgtccccccgcggacagccccgaggctggagagggagaaggggacggcggcgcggcgacgcacgaaggccctccccgcccatttccttcctgccggcgccgcaccgcttcgccccgcgcccgctagagggggtgcggcggcgcctcccagatttcggctccgcacagatttgggacaaaggaagtccctgcgccctctcgcacgattaccataaaaggcaatggctgcggctcgccgcgcctcgacagccgccggcgctccgggggccgccgcgcccctcccccgagccctccccggcccgaggcggccccgccccgcccggcacccccacctgccgccaccccccgcccggcacggcgagccccgcgccacgccccgtacggagccccgcacccgaagccgggccgtgctcagcaactcggggaggggggtgcagggggggttgcagcccgaccgacgcgcccacaccccctgctcacccccccacgcacacaccccgcacgcagcctttgttcccctcgcagccccccccgcaccgcggggcaccgcccccggccgcgctcccctcgcgcacactgcggagcgcacaaagccccgcgccgcgcccgcagcgctcacagccgccgggcagcgcggagccgcacgcggcgctccccacgcacacacacacgcacgcaccccccgagccgctccccccgcacaaagggccctcccggagcccctcaaggctttcacgcagccacagaaaagaaacaagccgtcattaaaccaagcgctaattacagcccggaggagaagggccgtcccgcccgctcacctgtgggagtaacgcggtcagtcagagccggggcgggcggcgcgaggcggcggcggagcggggcacggggcgaaggcagcgcgcagcgactcccgcccgccgcgcgcttcgctttttatagggccgccgccgccgccgcctcgccataaaaggaaactttcggagcgcgccgctctgattggctgccgccgcacctctccgcctcgccccgccccgcccctcgccccgccccgccccgcctggcgcgcgccccccccccccccgcccccatcgctgcacaaaataattaaaaaataaataaatacaaaattgggggtggggaggggggggagatggggagagtgaagcagaacgtggggctcacctcgaccatggtaatagcgatgactaatacgtagatgtactgccaagtaggaaagtcccataaggtcatgtactgggcataatgccaggcgggccatttaccgtcattgacgtcaatagggggcgtacttggcatatgatacacttgatgtactgccaagtgggcagtttaccgtaaatactccacccattgacgtcaatggaaagtccctattggcgttactatgggaacatacgtcattattgacgtcaatgggcgggggtcgttgggcggtcagccaggcgggccatttaccgtaagttatgtaacgcggaactccatatatgggctatgaactaatgaccccgtaattgattactattaataactagtcaataatcaat

SEQ ID NO: 6 - DNA, 48 bp, Artificial Sequence; identical to SEQ ID NO: 4
  polynucleotide

SEQ ID NO: 7 - DNA, 313 bp, Mus musculus
ctgcagcagctggcaggaagcaggtcatgtggcaaggctatttggggaagggaaaataaaaccactaggtaaacttgtagctgtggtttgaagaagtggttttgaaacactctgtccagccccaccaaaccgaaagtccaggctgagcaaaacaccacctgggtaatttgcatttctaaaataagttgaggattcagccgaaactggagaggtcctcttttaacttattgagttcaaccttttaattttagcttgagtagttctagtttccccaaacttaagtttatcgacttctaaaatgtatttagaattc

SEQ ID NO: 8 - DNA, 1000 bp, Artificial Sequence
  polynucleotide
ttaaaaaaaaaaaaaaaggaaagggacttctctgtgtttggcaacacaagtgcgatgcacaggcaggaagatcaaatctgtcccaacaatacaggggacagagggtcaacctacaaaaggaaagaacctggggcagtgtgaagacaacactgtagaagccaaggctgagttcactgagctctcgttagtgagactacacagcaaggaggtggcgggcactgagcagtgaggccccgggaagtgggggtgatggtggtgacggtggtaactgttaagaactgggggaaagaattgtggagaaccaagctaaatagttatgtcaaaccacatgtttaggagcctgggttgacttcatagggagtaggcatggaggctaatctagaggtttgtgtataggcaagaagtgaatcctgacccaagaatagagagtgctaaacggacttagttcaaagacaactgaaaaagacaatgcctgcaaaacaaagctaaggccagagctcttggactatgaagagttcagggaacctaagaacagggaccatctgtgtacaggccaaggccggtagaagcagcctaggaagtgtcaagagccaacgtggctgggtgggcaaagacaggaagggactgttaggctgcagggatgtgccgacttcaatgtgcttcagtattgtccagattgtgtgcagccatatggcccaggtataagaggtttaacagtggaacacagatgcccacatcagacagctggggggcgggggtgaacacagatacccatactggaaagcaggtggggcattttcctaggaacgggactgggctcaatggcctcaggtctcatctggtctggtgatcctgacattgataggcccaaatgttggatatcacctactccatgtagagagtcggggacatgggaagggtgcaaaagagcggccttctagaaggtttggtcctgtcctgtcctgtctgacagtgtaatcacatatactttttcttgtag

SEQ ID NO: 9 - DNA, 243 bp, Artificial Sequence
  polynucleotide
aagatcaaaagttgttcttctcccttctggagatttctatgtcctttacaactcaattggttaatatcctgggttggagtcccacacatcttgacaaacagagacaaatttgagtatcaccagccaaaagtcatacccaaaaacagcctggcatgaccacacaccagactcaaacttaccctacctttatcctggtggcttctcatctccagaccccagtaacacatagctttctctccacag

SEQ ID NO: 10 - DNA, 4252 bp, Artificial Sequence
  polynucleotide
tgcccagggattgtggttgtaagccttgcatatgtacaggtaagtcagtggccttcacctgacccagatgcaacaagtggcaatgttggagggtggccaggtattgacctatttccacctttcttcttcatccttagtcccagaagtatcatctgtcttcatcttccccccaaagcccaaggatgtgctcaccattactctgactcctaaggtcacgtgtgttgtggtagacatcagcaaggatgatcccgaggtccagttcagctggtttgtagatgatgtggaggtgcacacagctcagacgcaaccccgggaggagcagttcaacagcactttccgctcagtcagtgaacttcccatcatgcaccaggactggctcaatggcaaggagttcaaatgcagggtcaacagtgcagctttccctgcccccatcgagaaaaccatctccaaaaccaaaggtgagagctgcagtgtgtgacatagaagctgcaatagtcagtccatagacagagcttggcataacagacccctgccctgttcgtgacctctgtgctgaccaatctctttacccacccacaggcagaccgaaggctccacaggtgtacaccattccacctcccaaggagcagatggccaaggataaagtcagtctgacctgcatgataacagacttcttccctgaagacattactgtggagtggcagtggaatgggcagccagcggagaactacaagaacactcagcccatcatgaacacgaatggctcttacttcgtctacagcaagctcaatgtgcagaagagcaactgggaggcaggaaatactttcacctgctctgtgttacatgagggcctgcacaaccaccatactgagaagagcctctcccactctcctggtaaatgatcccagtgtccttggagccctctggtcctacaggactctgacacctacctccacccctccctgtataaataaagcacccagcactgccttgggaccctgcaataacgtcctggtgatttctgagatgtagagtctagctaggtcatggaatgaggggtctccatggtttgagccctgagttgtgactaaggaaaaactcataggcctacactgccacacccagcacttttgaatttgcctgacatgaaaagaatttacctctccctggaaagtggagccttatccctaggcagttcccttaccagaccttcctctagcttgcactatgttctgggcacagaatgtgtctaaccccccaaagtaaggaagacacaacctctacttccctcactctgtccttaccccttttcctggctaagcatctcactgagtgcgctgaatagatgcatgtggccacagcttgcagacagacctttgccatctctccgctcagctttccagaggctaagtctagcccgtatggtgatgatgcagggagctctatgctatctcagtgttatcagactcctaagtggaggatcaacatggtcccattaaaaccaacctgctcagcaacaccctgccaataaggcccgtatgtgaaaatgtgcacacatctacacatgcacaggcacacacacacacacatgcatgggcacacacacatacagagagagagaatcacagaaactcccatgagcatcctatacagtactcaaagataaaaaggtaccaggtctacccacatgatcatcctcggcatttacaagtgggccaactgatacagataaaacttttctatgccaaggacgccaacaaccttcctcatatacacaagtccgctcatgacaaatctgtccctgaacctcagactggcgcccgtgactcacacagtggacactcctccaaagctgtatagcttcctttacttccctgtgtgtactttctctgaagtacactcatcacacagaagaggccctgtgattactctggccctctgttcttggtcatcagagaatagacagaagatcaggcaaactacacagacacttcccacaatcatcacaggccctgactctgctctccagtctcaaaactgaaggctggagcacacagaaataagctcctacacagcccagaccagtatcgggtccagtgtgtctgaatgagcccagggacaaaatggcagcactttggggaactgagatttctggtccaagaaggagagatggaggcccagggagggtctgctgacccagcccagcccagcccagctgcagctttctcctgggcctccatgcagcttcctgccacacagggaatggccctagccccaccttattgggacaaacactgaccgccctctctgtccagggctgcaactggacgagacctgtgctgaggcccaggacggggagctggacgggctctggacgaccatcaccatcttcatcagcctcttcctgctcagcgtgtgctacagcgctgctgtcacactcttcaaggtcagccatactgtccccacagtgtctacaatgtcctcatactcttccccatactgtccctgtggtgacctataccccacactgtcccatgctaatgaccacagtcttacatgctatgtaatgctgtctacccttctgtatgcacagtctcacaatgtcccatgcagtctccacgatgctccatgctgccccttgttccacgctatgctgtcccatgctattgtctgtattttcatgctcttttcacactgtccctagtgtcacattctgcccatgttgtccaccacattgtccccactctgcacacagcctcacactgtaccctgctacccgataatgttccctgttgtccccaactctctccctgcatcatttgtcaactgtcccctgaattcccatgttgttcccacactgttagtgtgtaatgtgctctgtcccaggtgtaccttgttccgtgctgtctcacttcatcgcccattctgtccttttactaaccccactctatcaccacactgtccctatgcactgcccacattgtcctcatactgtcccattttgtatcttcatcctgtccccatagtgtccaatgatctaccccacactattcccacttcatgcccctacaatttccctattccatccctctctggtcaccatgccatccttcccactcctgcacagctggagagggactcccgggatgagtccttgcccagatgagctacctatctagaggagtcttcaggtgggaagggaatgcagtcttgatcttggtcttattcaccctgtctcacaggtaaagtggatcttctcctcggtggtggagctgaagcagacactggttcctgaatacaagaacatgattgggcaagcgccctaggccacctcttgtaatggcaggggatttcccaggccccaaaggaccctgtccaatatgccaagcagcacaactgagatcacactgtctgctcatctcgctttcctccgaccccgagactcagctactctcaaattttccctctctgaaggaccatgtggacattacattgctccaggccacagccaccaggacctaaaacaccatcacagcagcaccaaagacactggatagacccacaagagcaatagcttcctcaacagtatatccaaactgttgggacaaacgagcaatcactgaagaagtgacaagttcccacaatgtcagtgtccagctgagaaggggcaaaaagtggtaccagccctgtccacaccaccttctaattcacaggaatccgtgatagaagaggcaggttgtagatccgaaagatgagacagattttatcaactccagaaagagctgggcccaactgaatctaactgaattattctagcgaccttggcattgccatgacctgccatgaccttcctccttagcacttcgatgaaccctgggatatggaaaatgcctgtgtttctcagggtttgggaagaaccatccatgttgggattcttgtgtagatcctcctcctggtcacagatgcaatacactggattttcaggcaaaggagcaaattcacagacaactctggccctacagtcctcagacctagacaccaccatctccttggaattatcaaatctaacacccggcacacaacaaagaaggactgggactttgaggcctttgtgtagccctagagggggcagaggccactgagcagggattgggtgatcagcaaggacctcctggagagggacctgaggagcaggttccaattgggccaaagaaagaagaagaacaatagaggtgaaggatgctggaaagag

SEQ ID NO: 11 - DNA, 623 bp, Homo sapiens
gggtggcatccctgtgacccctccccagtgcctctcctggccctggaagttgccactccagtgcccaccagccttgtcctaataaaattaagttgcatcattttgtctgactaggtgtccttctataatattatggggtggaggggggtggtatggagcaaggggcaagttgggaagacaacctgtagggcctgcggggtctattgggaaccaagctggagtgcagtggcacaatcttggctcactgcaatctccgcctcctgggttcaagcgattctcctgcctcagcctcccgagttgttgggattccaggcatgcatgaccaggctcagctaatttttgtttttttggtagagacggggtttcaccatattggccaggctggtctccaactcctaatctcaggtgatctacccaccttggcctcccaaattgctgggattacaggcgtgaaccactgctcccttccctgtccttctgattttaaaataactataccagcaggaggacgtccagacacagcataggctacctggccatgcccaaccggtgggacatttgagttgcttgcttggcactgtcctctcatgcgttgggtccactcagtagatgcctgttgaatt

SEQ ID NO: 12 - DNA, 4565 bp, Artificial Sequence
  polynucleotide
gtgttcatgcccctagagttggctgaagggccagatccacctactctagaggcatctctccctgtctgtgaaggcttccaaagtcacgttcctgtggctagaaggcagctccatagccctgctgcagtttcgtcctgtataccaggttcacctactaccatatctagccctgcctgccttaagagtagcaacaaggaaatagcagggtgtagagggatctcctgtctgacaggaggcaagaagacagattcttacccctccatttctcttttatccctctctggtcctcagagagtcagtccttcccaaatgtcttccccctcgtctcctgcgagagccccctgtctgataagaatctggtggccatgggctgcctggcccgggacttcctgcccagcaccatttccttcacctgaaactaccagaacaacactgaagtcatccagggtatcagaaccttcccaacactgaggacagggggcaagtacctagccacctcgcaggtgttgctgtctcccaagagcatccttgaaggttcagatgaatacctggtatgcaaaatccactacggaggcaaaaacaaagatctgcatgtgcccattccaggtaagaaccaaaccctcccagcaggggtgcccaggcccaggcatggcccagagggagcagcggggtggggcttaggccaagctgagctcacaccttgacctttcattccagctgtcgcagagatgaaccccaatgtaaatgtgttcgtcccaccacgggatggcttctctggccctgcaccacgcaagtctaaactcatctgcgaggccacgaacttcactccaaaaccgatcacagtatcctgactaaaggatgggaagctcgtggaatctggcttcaccacagatccggtgaccatcgagaacaaaggatccacaccccaaacctacaaggtcataagcacacttaccatctctgaaatcgactggctgaacctgaatgtgtacacctgccgtgtggatcacaggggtctcaccttcttgaagaacgtgtcctccacatgtgctgccagtgagtggcctgggctaagcccaatgcctagccctcccagattagggaagtcctcctacaattatggccaatgccacccagacatggtcatttgctccttgaactttggctccccagagtggccaaggacaagaatgagcaataggcagtagaggggtgagaatcagctggaaggaccagcatcttcccttaagtaggtttgggggatggagactaagcttttttccaacttcacaactagatatgtcataacctgacacagtgttctcttgactgcaggtccctccacagacatcctaaccttcaccatccccccctcctttgccgacatcttcctcagcaagtccgctaacctgacctgtctggtctcaaacctggcaacctatgaaaccctgaatatctcctgagcttctcaaagtggtgaaccactggaaaccaaaattaaaatcatggaaagccatcccaatggcaccttcagtgctaagggtgtggctagtgtttgtgtggaagactggaataacaggaaggaatttgtgtgtactgtgactcacagggatctgccttcaccacagaagaaattcatctcaaaacccaatggtaggtatccccccttcccttcccctccaattgcaggacccttcctgtacctcatagggagggcaggtcctcttccaccctatcctcactactgtcttcatttacagaggtgcacaaacatccacctgctgtgtacctgctgccaccagctcgtgagcaactgaacctgagggagtcagccacagtcacctgcctggtgaagggcttctctcctgcagacatcagtgtgcagtggcttcagagagggcaactcttgccccaagagaagtatgtgaccagtgccccgatgccagagcctggggccccaggcttctactttacccacagcatcctgactgtgacagaggaggaatggaactccggagagacctatacctgtgttgtaggccacgaggccctgccacacctggtgaccgagaggaccgtggacaagtccactggtaaacccacactgtacaatgtctccctgatcatgtctgacacaggcggcacctgctattgaccatgctagcgctcaaccaggcaggccctgggtgtccagttgctctgtgtatgcaaactaaccatgtcagagtgagatgttgcattttataaaaattagaaataaaaaaaatccattcaaacgtcactggttttgattatacaatgctcatgcctgctgagacagttgtgttttgcttgctctgcacacaccctgcatacttgcctccaccctggcccttcctctaccttgccagtttcctccttgtgtgtgaactcagtcaggcttacaacagacagagtatgaacatgcgattcctccagctacttctagatatatggctgaaagcttgcctaacctggtgcaggcagcattcaggcacatatatagacacacatgcatttatacatagatatataggtacacatgtgtagacacatacatgaatgtgtattcatggacacacagacaaaggtacacatatatacacatgagttcatgcgcacacacatgcatggacacttacaaacgccttcagagacaaataggcatagacacacaaccactcacagaaacagataccaatatgcatggtcctgtgtacacagaaacagactataggcaaatatacacaaataaactatatagatacaaagatatgcatatacacacatgtacagaaacatcttcacatgtgtacactaacatgtgaacaggtatagcacacagatacacctggactctgaccagggctgtaatctccaaggctcacggctcagagagcctacactaggctgggtcactgatactcctcaggagcccactctatgattgggagagataaccccaggtacaaagtatgcctatctgtctcaacaccatggggcagaagatactccactaaccacccatgacagaaagttagccttggctgtgtctccattaatagaacacctcagaagaccaatgtgaaattgcctaacccactcacacccaccctgatctccagttcaaaatgcagaaaacataatgcagttgtccaaaagatgccccaaccacacacacacacacacacacacacacacacacacacacacacacacacacacacacacaccatcaaggagcctctgtaaggagtcaccacccaataacactgcctctttgggctcatatcctggacattcttcatattcatatccatttggggcctaggctttagatatccccaagggctcatctttacagggatcagagatcccaataaatgccctggtcccacagcctccctcaggtatctgtctgtttatctcttggtaccaagacccaacattgctggcaggggtaggacaagcaacgcacgggaactctgatcaaagaaagtcatgagatgcctgagtccttcaggaagtaaggagggacaacctctggtatccctgttcttattgctaaagcccaagagacagggagacctgctctaaattctcagtctaaacagcaccgatggcaccacctgctcagggaaagtccagagcacaccaatatcattttgccacagttcctgagtctgcctttacccaggtccatacattgcatctgtcttgcttgctctgctgccccagggctcctggaacaaaggctccaaattagtgtgtcctacagcttggcctgttctgtgcctccgtctagcttgagctattaggggaccagtcaatactcgctaagattctccagaaccatcagggcaccccaacccttatgcaaatgctcagtcaccccaagacttggcttgaccctccctctctgtgtcccttcatagagggggaggtgaatgctgaggaggaaggctttgagaacctgtggaccactgcctccaccttcatcgtcctcttcctcctgagcctcttctacagcaccaccgtcaccctgttcaaggtagtgtggttgtggggctgaggacacagggctgggacagggagtcaccagtcctcactgcctctacctctactccctacaagtggacagcaattcacactgtctctgtcacctgcaggtgaaatgactctcagcatggaaggacagcagagaccaagagatcctcccacagggacactacctctgggcctgggatacctgactgtatgactagtaaacttattcttacgtctttcctgtgttgccctccagcttttatctctgagatggtcttctttctagactgaccaaagactttttgtcaacttgtacaatctgaagcaatgtctggcccacagacagctgagctgtaaacaaatgtcacatggaaataaatactttatcttgtgaactcactttattgtgaaggaatttgttttgtttttcaaacctttcctgcggtgttgacagcccaaggattatctgaatagagcttaggaactggaaatggaacagt

SEQ ID NO: 13 - DNA, 291 bp, Artificial Sequence
  polynucleotide
gtgttcatgcccctagagttggctgaagggccagatccacctactctagaggcatctctccctgtctgtgaaggcttccaaagtcacgttcctgtggctagaaggcagctccatagccctgctgcagtttcgtcctgtataccaggttcacctactaccatatctagccctgcctgccttaagagtagcaacaaggaaatagcagggtgtagagggatctcctgtctgacaggaggcaagaagacagattcttacccctccatttctcttttatccctctctggtcctcag

SEQ ID NO: 14 - DNA, 4227 bp, Mus musculus
agagtcagtccttcccaaatgtcttccccctcgtctcctgcgagagccccctgtctgataagaatctggtggccatgggctgcctggcccgggacttcctgcccagcaccatttccttcacctgaaactaccagaacaacactgaagtcatccagggtatcagaaccttcccaacactgaggacagggggcaagtacctagccacctcgcaggtgttgctgtctcccaagagcatccttgaaggttcagatgaatacctggtatgcaaaatccactacggaggcaaaaacaaagatctgcatgtgcccattccaggtaagaaccaaaccctcccagcaggggtgcccaggcccaggcatggcccagagggagcagcggggtggggcttaggccaagctgagctcacaccttgacctttcattccagctgtcgcagagatgaaccccaatgtaaatgtgttcgtcccaccacgggatggcttctctggccctgcaccacgcaagtctaaactcatctgcgaggccacgaacttcactccaaaaccgatcacagtatcctgactaaaggatgggaagctcgtggaatctggcttcaccacagatccggtgaccatcgagaacaaaggatccacaccccaaacctacaaggtcataagcacacttaccatctctgaaatcgactggctgaacctgaatgtgtacacctgccgtgtggatcacaggggtctcaccttcttgaagaacgtgtcctccacatgtgctgccagtgagtggcctgggctaagcccaatgcctagccctcccagattagggaagtcctcctacaattatggccaatgccacccagacatggtcatttgctccttgaactttggctccccagagtggccaaggacaagaatgagcaataggcagtagaggggtgagaatcagctggaaggaccagcatcttcccttaagtaggtttgggggatggagactaagcttttttccaacttcacaactagatatgtcataacctgacacagtgttctcttgactgcaggtccctccacagacatcctaaccttcaccatccccccctcctttgccgacatcttcctcagcaagtccgctaacctgacctgtctggtctcaaacctggcaacctatgaaaccctgaatatctcctgagcttctcaaagtggtgaaccactggaaaccaaaattaaaatcatggaaagccatcccaatggcaccttcagtgctaagggtgtggctagtgtttgtgtggaagactggaataacaggaaggaatttgtgtgtactgtgactcacagggatctgccttcaccacagaagaaattcatctcaaaacccaatggtaggtatccccccttcccttcccctccaattgcaggacccttcctgtacctcatagggagggcaggtcctcttccaccctatcctcactactgtcttcatttacagaggtgcacaaacatccacctgctgtgtacctgctgccaccagctcgtgagcaactgaacctgagggagtcagccacagtcacctgcctggtgaagggcttctctcctgcagacatcagtgtgcagtggcttcagagagggcaactcttgccccaagagaagtatgtgaccagtgccccgatgccagagcctggggccccaggcttctactttacccacagcatcctgactgtgacagaggaggaatggaactccggagagacctatacctgtgttgtaggccacgaggccctgccacacctggtgaccgagaggaccgtggacaagtccactggtaaacccacactgtacaatgtctccctgatcatgtctgacacaggcggcacctgctattgaccatgctagcgctcaaccaggcaggccctgggtgtccagttgctctgtgtatgcaaactaaccatgtcagagtgagatgttgcattttataaaaattagaaataaaaaaaatccattcaaacgtcactggttttgattatacaatgctcatgcctgctgagacagttgtgttttgcttgctctgcacacaccctgcatacttgcctccaccctggcccttcctctaccttgccagtttcctccttgtgtgtgaactcagtcaggcttacaacagacagagtatgaacatgcgattcctccagctacttctagatatatggctgaaagcttgcctaacctggtgcaggcagcattcaggcacatatatagacacacatgcatttatacatagatatataggtacacatgtgtagacacatacatgaatgtgtattcatggacacacagacaaaggtacacatatatacacatgagttcatgcgcacacacatgcatggacacttacaaacgccttcagagacaaataggcatagacacacaaccactcacagaaacagataccaatatgcatggtcctgtgtacacagaaacagactataggcaaatatacacaaataaactatatagatacaaagatatgcatatacacacatgtacagaaacatcttcacatgtgtacactaacatgtgaacaggtatagcacacagatacacctggactctgaccagggctgtaatctccaaggctcacggctcagagagcctacactaggctgggtcactgatactcctcaggagcccactctatgattgggagagataaccccaggtacaaagtatgcctatctgtctcaacaccatggggcagaagatactccactaaccacccatgacagaaagttagccttggctgtgtctccattaatagaacacctcagaagaccaatgtgaaattgcctaacccactcacacccaccctgatctccagttcaaaatgcagaaaacataatgcagttgtccaaaagatgccccaaccacacacacacacacacacacacacacacacacacacacacacacacacacacacacacaccatcaaggagcctctgtaaggagtcaccacccaataacactgcctctttgggctcatatcctggacattcttcatattcatatccatttggggcctaggctttagatatccccaagggctcatctttacagggatcagagatcccaataaatgccctggtcccacagcctccctcaggtatctgtctgtttatctcttggtaccaagacccaacattgctggcaggggtaggacaagcaacgcacgggaactctgatcaaagaaagtcatgagatgcctgagtccttcaggaagtaaggagggacaacctctggtatccctgttcttattgctaaagcccaagagacagggagacctgctctaaattctcagtctaaacagcaccgatggcaccacctgctcagggaaagtccagagcacaccaatatcattttgccacagttcctgagtctgcctttacccaggtccatacattgcatctgtcttgcttgctctgctgccccagggctcctggaacaaaggctccaaattagtgtgtcctacagcttggcctgttctgtgcctccgtctagcttgagctattaggggaccagtcaatactcgctaagattctccagaaccatcagggcaccccaacccttatgcaaatgctcagtcaccccaagacttggcttgaccctccctctctgtgtcccttcatagagggggaggtgaatgctgaggaggaaggctttgagaacctgtggaccactgcctccaccttcatcgtcctcttcctcctgagcctcttctacagcaccaccgtcaccctgttcaaggtagtgtggttgtggggctgaggacacagggctgggacagggagtcaccagtcctcactgcctctacctctactccctacaagtggacagcaattcacactgtctctgtcacctgcaggtgaaatgactctcagcatggaaggacagcagagaccaagagatcctcccacagggacactacctctgggcctgggatacctgactgtatgactagtaaacttattcttacgtctttcctgtgttgccctccagcttttatctctgagatggtcttctttctagactgaccaaagactttttgtcaacttgtacaatctgaagcaatgtctggcccacagacagctgagctgtaaacaaatgtcacatggaaataaatactttatcttgtgaactcactttattgtgaaggaatttgttttgtttttcaaacctttcctgcggtgttgaca

SEQ ID NO: 15 - DNA, 46 bp, Artificial Sequence
  polynucleotide
gcccaaggattatctgaatagagcttaggaactggaaatggaacag

SEQ ID NO: 16 - DNA, 294 bp, Homo sapiens
cctccaccaagggcccatcggtcttccccctggcaccctcctccaagagcacctctgggggcacagcagccctgggctgcctggtcaaggactacttccccgaaccggtgacggtgtcgtggaactcaggcgccctgaccagcggcgtgcacaccttcccggctgtcctacagtcctcaggactctactccctcagcagcgtggtgaccgtgccctccagcagcttgggcacccagacctacatctgcaacgtgaatcacaagcccagcaacaccaaggtggacaagaaagttg

SEQ ID NO: 17 - DNA, 330 bp, Homo sapiens
cacctgaactcctggggggaccgtcagtcttcctcttccccccaaaacccaaggacaccctcatgatctcccggacccctgaggtcacatgcgtggtggtggacgtgagccacgaagaccctgaggtcaagttcaactggtacgtggacggcgtggaggtgcataatgccaagacaaagccgcgggaggagcagtacaacagcacgtaccgtgtggtcagcgtcctcaccgtcctgcaccaggactggctgaatggcaaggagtacaagtgcaaggtctccaacaaagccctcccagcccccatcgagaaaaccatctccaaagccaaag

SEQ ID NO: 18 - DNA, 320 bp, Homo sapiens
ggcagccccgagaaccacaggtgtacaccctgcccccatcccgggatgagctgaccaagaaccaggtcagcctgacctgcctggtcaaaggcttctatcccagcgacatcgccgtggagtgggagagcaatgggcagccggagaacaactacaagaccacgcctcccgtgctggactccgacggctccttcttcctctacagcaagctcaccgtggacaagagcaggtggcagcaggggaacgtcttctcatgctccgtgatgcatgaggctctgcacaaccactacacacagaagagcctctccctgtctccgggtaaa